European Patent Application EP 4 772 248 A2, published July 8, 2026. Title: USE OF C/EBP-BETA ANTAGONIST AND IMMUNOMODULATOR. Applicant: SAPIENCE THERAPEUTICS,INC. Application EP. The sequence listing filed with the application follows.

SEQUENCE LISTING (3 sequences)

SEQ ID NO: 1 - protein, 22 aa, synthetic construct
  REGION 1..22: note = D-Amino acid residues
VAEAREELERLEARLGQARGEL

SEQ ID NO: 2 - protein, 38 aa, synthetic construct
  REGION 1..38: note = D-Amino acid residues
VAEAREELERLEARLGQARGELKKWKMRRNQFWLKLQR

SEQ ID NO: 3 - protein, 22 aa, synthetic construct
LEGRAQGLRAELRELEERAEAV